European Patent Application EP 4 242 231 A1, published September 13, 2023. Title: ANTI-SIGLEC-15 ANTIBODY AND USES THEREOF IN PREPARING DRUGS. Applicant: SHANGHAI JMT-BIO TECHNOLOGY CO., LTD. Application EP21888626.5. The sequence listing filed with the application follows.

SEQUENCE LISTING (82 sequences)

SEQ ID NO: 1 - protein, 5 aa, Artificial Sequence
  21F6C6 HCDR1
SYAMS

SEQ ID NO: 2 - protein, 17 aa, Artificial Sequence
  21F6C6 HCDR2
TISSGGSLIYYPDSVTG

SEQ ID NO: 3 - protein, 17 aa, Artificial Sequence
  21F6C6-hVH2 HCDR2
TISSGGSLIYYADSVTG

SEQ ID NO: 4 - protein, 17 aa, Artificial Sequence
  21F6C6-hVH3/hVH4 HCDR2
TISSGGSLIYYADSVKG

SEQ ID NO: 5 - protein, 16 aa, Artificial Sequence
  21F6C6 HCDR3
HGYYYGDSTLYYAMDY

SEQ ID NO: 6 - protein, 15 aa, Artificial Sequence
  21F6C6 LCDR1
KASQSVDYDGDSYMN

SEQ ID NO: 7 - protein, 15 aa, Artificial Sequence
  21F6C6-hVL1~4 LCDR1
RASQSVDYDGDSYMN

SEQ ID NO: 8 - protein, 7 aa, Artificial Sequence
  21F6C6 LCDR2
AASNLES

SEQ ID NO: 9 - protein, 7 aa, Artificial Sequence
  21F6C6-hVL4 LCDR2
AASNLQS

SEQ ID NO: 10 - protein, 9 aa, Artificial Sequence
  21F6C6 LCDR3
QQSNEAPLT

SEQ ID NO: 11 - protein, 5 aa, Artificial Sequence
  75E1F2 HCDR1
DYGMH

SEQ ID NO: 12 - protein, 17 aa, Artificial Sequence
  75E1F2 HCDR2
YISSGSSIIDYSDTVKG

SEQ ID NO: 13 - protein, 9 aa, Artificial Sequence
  75E1F2 HCDR3
REDHYAMDY

SEQ ID NO: 14 - protein, 11 aa, Artificial Sequence
  75E1F2 LCDR1
KASQDVYTAVA

SEQ ID NO: 15 - protein, 7 aa, Artificial Sequence
  75E1F2 LCDR2
SASYRFT

SEQ ID NO: 16 - protein, 9 aa, Artificial Sequence
  75E1F2 LCDR3
QQHYSTPWT

SEQ ID NO: 17 - protein, 5 aa, Artificial Sequence
  124B11F6 HCDR1
DYYMH

SEQ ID NO: 18 - protein, 17 aa, Artificial Sequence
  124B11F6 HCDR2
RIDPEDDKTKYAPKFQG

SEQ ID NO: 19 - protein, 17 aa, Artificial Sequence
  124B11F6-hVH4 HCDR2
RIDPEDDKTKYSQKFQG

SEQ ID NO: 20 - protein, 9 aa, Artificial Sequence
  124B11F6 HCDR3
GWLGYIMDF

SEQ ID NO: 21 - protein, 12 aa, Artificial Sequence
  124B11F6 LCDR1
TLSSQHSTYTID

SEQ ID NO: 22 - protein, 11 aa, Artificial Sequence
  124B11F6 LCDR2
LKEDGSHSTGD

SEQ ID NO: 23 - protein, 11 aa, Artificial Sequence
  124B11F6-hVL3~4 LCDR2
LKEDGSHSKGD

SEQ ID NO: 24 - protein, 13 aa, Artificial Sequence
  124B11F6 LCDR3
GVGATIKEQFVYV

SEQ ID NO: 25 - protein, 5 aa, Artificial Sequence
  174C11C9 HCDR1
DYYMN

SEQ ID NO: 26 - protein, 17 aa, Artificial Sequence
  174C11C9 HCDR2
VFNPYSGGISYNQKFKG

SEQ ID NO: 27 - protein, 17 aa, Artificial Sequence
  174C11C9-hVH3 HCDR2
VFNPYSGGISYAQKFKG

SEQ ID NO: 28 - protein, 17 aa, Artificial Sequence
  174C11C9-hVH4 HCDR2
VFNPYSGGISYAQKFQG

SEQ ID NO: 29 - protein, 15 aa, Artificial Sequence
  174C11C9 HCDR3
DYYYLSSHGFYALDY

SEQ ID NO: 30 - protein, 15 aa, Artificial Sequence
  174C11C9 LCDR1
RASESVDSYGNSFIH

SEQ ID NO: 31 - protein, 15 aa, Artificial Sequence
  174C11C9-hVL4 LCDR1
RASESVDSYGNTFIH

SEQ ID NO: 32 - protein, 7 aa, Artificial Sequence
  174C11C9 LCDR2
RASNLES

SEQ ID NO: 33 - protein, 7 aa, Artificial Sequence
  174C11C9-hVL4 LCDR2
RASNLQS

SEQ ID NO: 34 - protein, 9 aa, Artificial Sequence
  174C11C9 LCDR3
QQSNEDPLT

SEQ ID NO: 35 - protein, 5 aa, Artificial Sequence
  255C12B10 HCDR1
GYNMN

SEQ ID NO: 36 - protein, 17 aa, Artificial Sequence
  255C12B10 HCDR2
YINPNNGGTRYNQKFKG

SEQ ID NO: 37 - protein, 6 aa, Artificial Sequence
  255C12B10 HCDR3
DYGIDY

SEQ ID NO: 38 - protein, 11 aa, Artificial Sequence
  255C12B10 LCDR1
QATQDIVKNLN

SEQ ID NO: 39 - protein, 7 aa, Artificial Sequence
  255C12B10 LCDR2
YATELAE

SEQ ID NO: 40 - protein, 9 aa, Artificial Sequence
  255C12B10 LCDR3
LQFYEFPYT

SEQ ID NO: 41 - protein, 125 aa, Artificial Sequence
  21F6C6 Heavy Chain Variable Region
EVMLVESGGGLVKPGGSLKLSCAASGFTFSSYAMSWVRQSPEKRLEWVATISSGGSLIYYPDSVTGRFTISRDNAKSTLYLQMSSLRSEDTAMYYCVRHGYYYGDSTLYYAMDYWGPGTSVTVSS

SEQ ID NO: 42 - protein, 111 aa, Artificial Sequence
  21F6C6 Light Chain Variable Region
DIVLTQSPASLAVSLGQRATISCKASQSVDYDGDSYMNWYQQKPGQPPKLLIYAASNLESGIPARFSGSGSGTDFTLNIHPVEEEDAATYYCQQSNEAPLTFGAGTKLELK

SEQ ID NO: 43 - protein, 118 aa, Artificial Sequence
  75E1F2 Heavy Chain Variable Region
EVQLVESGGGSVKPGGSLKLSCAASGFTFSDYGMHWVRQAPEKGLEWITYISSGSSIIDYSDTVKGRFTISRDNAKDTLFLQMTSLRSEDTAIYYCVRREDHYAMDYWGQGTSVTVSS

SEQ ID NO: 44 - protein, 107 aa, Artificial Sequence
  75E1F2 Light Chain Variable Region
DIVMTQSHKFLSTSVGDRVSITCKASQDVYTAVAWFQQKPGQSPKLLFYSASYRFTGVPDRFNGSGSGTDFTLTITSMQAEDLAVYYCQQHYSTPWTFGGGTKLEIK

SEQ ID NO: 45 - protein, 118 aa, Artificial Sequence
  124B11F6 Heavy Chain Variable Region
EVQLQQSGAELVRPGASVKLSCTASVFNIKDYYMHWVKQRTEQGLEWIGRIDPEDDKTKYAPKFQGKATITADTSSNTAYLHLSTLTSEDTAVYYCVRGWLGYIMDFWGQGTSVTVSS

SEQ ID NO: 46 - protein, 115 aa, Artificial Sequence
  124B11F6 Light Chain Variable Region
QLVLTQSSSASFSLGASAKLTCTLSSQHSTYTIDWYQQQPLKPPKYVMELKEDGSHSTGDGIPDRFSGSSSGADRYLGISNIQPEDEAVYICGVGATIKEQFVYVFGGGTKVTVL

SEQ ID NO: 47 - protein, 124 aa, Artificial Sequence
  174C11C9 Heavy Chain Variable Region
EVQLQQSGPVLVKPGASVKMSCEASGYIFTDYYMNWVKQSPGKSLEWIGVFNPYSGGISYNQKFKGKATLTVDTSSSTAYMELNSLTSEDSAVYYCARDYYYLSSHGFYALDYWGQGTSVTVSS

SEQ ID NO: 48 - protein, 111 aa, Artificial Sequence
  174C11C9 Light Chain Variable Region
DIVLTQSPASLAVSLGQRATISCRASESVDSYGNSFIHWYQQRPGRPPKLLMYRASNLESGIPARFSGSGSRTDFTLTIDPVEADDVATYYCQQSNEDPLTFGAGTKLELK

SEQ ID NO: 49 - protein, 115 aa, Artificial Sequence
  255C12B10 Heavy Chain Variable Region
EVQLQQSGPELVKPGASVKMSCKASGYTFTGYNMNWVKQSHGKSLEWIGYINPNNGGTRYNQKFKGKATLTINKSSSTAYMELRSLTSEDSAVYYCARDYGIDYWGQGTTLTVSS

SEQ ID NO: 50 - protein, 107 aa, Artificial Sequence
  255C12B10 Light Chain Variable Region
EIQMTQSPSSMSASLGDRITITCQATQDIVKNLNWYQQKPGKPPSFLIYYATELAEGVPSRFSGSGSGSDYSLTISNLESEDFADYYCLQFYEFPYTFGGGTKLEIK

SEQ ID NO: 51 - protein, 125 aa, Artificial Sequence
  21F6C6-hVH1 Heavy Chain Variable Region
EVQLVESGGGLVKPGGSLRLSCAASGFTFSSYAMSWVRQAPGKGLEWVATISSGGSLIYYPDSVTGRFTISRDNAKSTLYLQMNSLRAEDTAVYYCVRHGYYYGDSTLYYAMDYWGQGTTVTVSS

SEQ ID NO: 52 - protein, 111 aa, Artificial Sequence
  21F6C6-hVL1 Light Chain Variable Region
DIQLTQSPSSLSASVGDRATITCRASQSVDYDGDSYMNWYQQKPGKAPKLLIYAASNLESGIPARFSGSGSGTDFTLTISSVQPEDFATYYCQQSNEAPLTFGQGTKLEIK

SEQ ID NO: 53 - protein, 125 aa, Artificial Sequence
  21F6C6-hVH2 Heavy Chain Variable Region
EVQLVESGGGLVKPGGSLRLSCAASGFTFSSYAMSWVRQAPGKGLEWVATISSGGSLIYYADSVTGRFTISRDNAKNTLYLQMNSLRAEDTAVYYCVRHGYYYGDSTLYYAMDYWGQGTTVTVSS

SEQ ID NO: 54 - protein, 111 aa, Artificial Sequence
  21F6C6-hVL2 Light Chain Variable Region
DIQLTQSPSSLSASVGDRATITCRASQSVDYDGDSYMNWYQQKPGKAPKLLIYAASNLESGVPSRFSGSGSGTDFTLTISSVQPEDFATYYCQQSNEAPLTFGQGTKLEIK

SEQ ID NO: 55 - protein, 125 aa, Artificial Sequence
  21F6C6-hVH3 Heavy Chain Variable Region
EVQLVESGGGLVKPGGSLRLSCAASGFTFSSYAMSWVRQAPGKGLEWVATISSGGSLIYYADSVKGRFTISRDNAKNTLYLQMNSLRAEDTAVYYCARHGYYYGDSTLYYAMDYWGQGTTVTVSS

SEQ ID NO: 56 - protein, 111 aa, Artificial Sequence
  21F6C6-hVL3 Light Chain Variable Region
DIQLTQSPSSLSASVGDRVTITCRASQSVDYDGDSYMNWYQQKPGKAPKLLIYAASNLESGVPSRFSGSGSGTDFTLTISSLQPEDFATYYCQQSNEAPLTFGQGTKLEIK

SEQ ID NO: 57 - protein, 125 aa, Artificial Sequence
  21F6C6-hVH4 Heavy Chain Variable Region
EVQLVESGGGLVKPGGSLRLSCAASGFTFSSYAMSWVRQAPGKGLEWVATISSGGSLIYYADSVKGRFTISRDNAKNSLYLQMNSLRAEDTAVYYCARHGYYYGDSTLYYAMDYWGQGTTVTVSS

SEQ ID NO: 58 - protein, 111 aa, Artificial Sequence
  21F6C6-hVL4 Light Chain Variable Region
DIQMTQSPSSLSASVGDRVTITCRASQSVDYDGDSYMNWYQQKPGKAPKLLIYAASNLQSGVPSRFSGSGSGTDFTLTISSLQPEDFATYYCQQSNEAPLTFGQGTKLEIK

SEQ ID NO: 59 - protein, 118 aa, Artificial Sequence
  124B11F6-hVH1 Heavy Chain Variable Region
QVQLVQSGAEVKKPGASVKVSCKASVFNIKDYYMHWVRQAPGQGLEWIGRIDPEDDKTKYAPKFQGRATITADTSTNTAYLELSSLRSEDTAVYYCVRGWLGYIMDFWGQGTTVTVSS

SEQ ID NO: 60 - protein, 115 aa, Artificial Sequence
  124B11F6-hVL1 Light Chain Variable Region
QLVLTQSPSASFSLGASAKLTCTLSSQHSTYTIDWYQQQPEKGPRYVMELKEDGSHSTGDGIPDRFSGSSSGAERYLTISSIQSEDEADYICGVGATIKEQFVYVFGGGTKVTVL

SEQ ID NO: 61 - protein, 118 aa, Artificial Sequence
  124B11F6-hVH2 Heavy Chain Variable Region
QVQLVQSGAEVKKPGASVKVSCKASVFNIKDYYMHWVRQAPGQGLEWIGRIDPEDDKTKYAPKFQGRVTITADTSTSTAYLELSSLRSEDTAVYYCVRGWLGYIMDFWGQGTTVTVSS

SEQ ID NO: 62 - protein, 115 aa, Artificial Sequence
  124B11F6-hVL2 Light Chain Variable Region
QLVLTQSPSASASLGASVKLTCTLSSQHSTYTIDWYQQQPEKGPRYVMELKEDGSHSTGDGIPDRFSGSSSGAERYLTISSLQSEDEADYICGVGATIKEQFVYVFGGGTKVTVL

SEQ ID NO: 63 - protein, 118 aa, Artificial Sequence
  124B11F6-hVH3 Heavy Chain Variable Region
QVQLVQSGAEVKKPGASVKVSCKASVFNIKDYYMHWVRQAPGQGLEWIGRIDPEDDKTKYAPKFQGRVTITRDTSASTAYMELSSLRSEDTAVYYCVRGWLGYIMDFWGQGTTVTVSS

SEQ ID NO: 64 - protein, 115 aa, Artificial Sequence
  124B11F6-hVL3 Light Chain Variable Region
QLVLTQSPSASASLGASVKLTCTLSSQHSTYTIDWYQQQPEKGPRYLMELKEDGSHSKGDGIPDRFSGSSSGAERYLTISSLQSEDEADYICGVGATIKEQFVYVFGGGTKVTVL

SEQ ID NO: 65 - protein, 118 aa, Artificial Sequence
  124B11F6-hVH4 Heavy Chain Variable Region
QVQLVQSGAEVKKPGASVKVSCKASVFNIKDYYMHWVRQAPGQGLEWIGRIDPEDDKTKYSQKFQGRVTITRDTSASTAYMELSSLRSEDTAVYYCARGWLGYIMDFWGQGTTVTVSS

SEQ ID NO: 66 - protein, 115 aa, Artificial Sequence
  124B11F6-hVL4 Light Chain Variable Region
QLVLTQSPSASASLGASVKLTCTLSSQHSTYTIDWHQQQPEKGPRYLMELKEDGSHSKGDGIPDRFSGSSSGAERYLTISSLQSEDEADYICGVGATIKEQFVYVFGGGTKVTVL

SEQ ID NO: 67 - protein, 124 aa, Artificial Sequence
  174C11C9-hVH1 Heavy Chain Variable Region
QVQLVQSGAEVKKPGASVKVSCKASGYIFTDYYMNWVRQAPGQGLEWIGVFNPYSGGISYNQKFKGRATLTVDTSTSTAYMELSSLRSEDTAVYYCARDYYYLSSHGFYALDYWGQGTTVTVSS

SEQ ID NO: 68 - protein, 111 aa, Artificial Sequence
  174C11C9-hVL1 Light Chain Variable Region
DIQLTQSPSSLSASVGDRATITCRASESVDSYGNSFIHWYQQKPGKAPKLLMYRASNLESGIPSRFSGSGSRTDFTLTISSVQPEDFATYYCQQSNEDPLTFGQGTKLEIK

SEQ ID NO: 69 - protein, 124 aa, Artificial Sequence
  174C11C9-hVH2 Heavy Chain Variable Region
QVQLVQSGAEVKKPGASVKVSCKASGYIFTDYYMNWVRQAPGQGLEWIGVFNPYSGGISYNQKFKGRVTLTVDTSTSTAYMELSSLRSEDTAVYYCARDYYYLSSHGFYALDYWGQGTTVTVSS

SEQ ID NO: 70 - protein, 111 aa, Artificial Sequence
  174C11C9-hVL2 Light Chain Variable Region
DIQLTQSPSSLSASVGDRVTITCRASESVDSYGNSFIHWYQQKPGKAPKLLMYRASNLESGIPSRFSGSGSGTDFTLTISSLQPEDFATYYCQQSNEDPLTFGQGTKLEIK

SEQ ID NO: 71 - protein, 124 aa, Artificial Sequence
  174C11C9-hVH3 Heavy Chain Variable Region
QVQLVQSGAEVKKPGASVKVSCKASGYIFTDYYMNWVRQAPGQGLEWIGVFNPYSGGISYAQKFKGRVTLTVDTSTSTAYMELSSLRSEDTAVYYCARDYYYLSSHGFYALDYWGQGTTVTVSS

SEQ ID NO: 72 - protein, 111 aa, Artificial Sequence
  174C11C9-hVL3 Light Chain Variable Region
DIQLTQSPSSLSASVGDRVTITCRASESVDSYGNSFIHWYQQKPGKAPKLLMYRASNLESGVPSRFSGSGSGTDFTLTISSLQPEDFATYYCQQSNEDPLTFGQGTKLEIK

SEQ ID NO: 73 - protein, 124 aa, Artificial Sequence
  174C11C9-hVH4 Heavy Chain Variable Region
QVQLVQSGAEVKKPGASVKVSCKASGYIFTDYYMNWVRQAPGQGLEWIGVFNPYSGGISYAQKFQGRVTMTRDTSTSTAYMELSSLRSEDTAVYYCARDYYYLSSHGFYALDYWGQGTTVTVSS

SEQ ID NO: 74 - protein, 111 aa, Artificial Sequence
  174C11C9-hVL4 Light Chain Variable Region
DIQMTQSPSSLSASVGDRVTITCRASESVDSYGNTFIHWYQQKPGKAPKLLMYRASNLQSGVPSRFSGSGSGTDFTLTISSLQPEDFATYYCQQSNEDPLTFGQGTKLEIK

SEQ ID NO: 75 - protein, 263 aa, Artificial Sequence
  hSiglec-15 Extracellular Domain
MEKSIWLLACLAWVLPTGSFVRTKIDTTENLLNTEVHSSPAQRWSMQVPPEVSAEAGDAAVLPCTFTHPHRHYDGPLTAIWRAGEPYAGPQVFRCAAARGSELCQTALSLHGRFRLLGNPRRNDLSLRVERLALADDRRYFCRVEFAGDVHDRYESRHGVRLHVTAAPRIVNISVLPSPAHAFRALCTAEGEPPPALAWSGPALGNSLAAVRSPREGHGHLVTAELPALTHDGRYTCTAANSLGRSEASVYLFRFHGASGAST

SEQ ID NO: 76 - protein, 483 aa, Artificial Sequence
  hS15-hFc Protein
FVRTKIDTTENLLNTEVHSSPAQRWSMQVPPEVSAEAGDAAVLPCTFTHPHRHYDGPLTAIWRAGEPYAGPQVFRCAAARGSELCQTALSLHGRFRLLGNPRRNDLSLRVERLALADDRRYFCRVEFAGDVHDRYESRHGVRLHVTAAPRIVNISVLPSPAHAFRALCTAEGEPPPALAWSGPALGNSLAAVRSPREGHGHLVTAELPALTHDGRYTCTAANSLGRSEASVYLFRFHGASGASTGGGSGGGSPKSSDKTHTCPPCPAPELLGGPSVFLFPPKPKDTLMISRTPEVTCVVVDVSHEDPEVKFNWYVDGVEVHNAKTKPREEQYNSTYRVVSVLTVLHQDWLNGKEYKCKVSNKALPAPIEKTISKAKGQPREPQVYTLPPSRDELTKNQVSLTCLVKGFYPSDIAVEWESNGQPENNYKTTPPVLDSDGSFFLYSKLTVDKSRWQQGNVFSCSVMHEALHNHYTQKSLSLSPGK

SEQ ID NO: 77 - protein, 390 aa, Artificial Sequence
  hS15-D1-hFc
PTGSFVRTKIDTTENLLNTEVHSSPAQRWSMQVPPEVSAEAGDAAVLPCTFTHPHRHYDGPLTAIWRAGEPYAGPQVFRCAAARGSELCQTALSLHGRFRLLGNPRRNDLSLRVERLALADDRRYFCRVEFAGDVHDRYESRHGVRLHVTAADIEGRMDPKSCDKTHTCPPCPAPELLGGPSVFLFPPKPKDTLMISRTPEVTCVVVDVSHEDPEVKFNWYVDGVEVHNAKTKPREEQYNSTYRVVSVLTVLHQDWLNGKEYKCKVSNKALPAPIEKTISKAKGQPREPQVYTLPPSRDELTKNQVSLTCLVKGFYPSDIAVEWESNGQPENNYKTTPPVLDSDGSFFLYSKLTVDKSRWQQGNVFSCSVMHEALHNHYTQKSLSLSPGK

SEQ ID NO: 78 - protein, 262 aa, Artificial Sequence
  hS15-His Protein
FVRTKIDTTENLLNTEVHSSPAQRWSMQVPPEVSAEAGDAAVLPCTFTHPHRHYDGPLTAIWRAGEPYAGPQVFRCAAARGSELCQTALSLHGRFRLLGNPRRNDLSLRVERLALADDRRYFCRVEFAGDVHDRYESRHGVRLHVTAAPRIVNISVLPSPAHAFRALCTAEGEPPPALAWSGPALGNSLAAVRSPREGHGHLVTAELPALTHDGRYTCTAANSLGRSEASVYLFRFHGASGASTGGGSGGGSHHHHHHHHHH

SEQ ID NO: 79 - protein, 262 aa, Artificial Sequence
  Cynomolgus Monkey S15-His Protein
FVRTKIDTTENLLNTEVHSSPAQRWSMQVPAEVSAAAGDAAVLPCTFTHPHRHYDGPLTAIWRAGEPYAGPQVFRCAAARGSELCQTALSLHGRFRLLGNPRRNDLSLRVERLALADDRRYFCRVEFAGDVHDRYESRHGVRLHVTAAPRIINISVLPGPAHAFRALCTAEGEPPPALAWSGPALGNGSAAVPSSGQGHGHLVTAELPALNHDGRYTCTAANSLGRSEASVYLFRFHGASGASTGGGSGGGSHHHHHHHHHH

SEQ ID NO: 80 - protein, 257 aa, Artificial Sequence
  mouse S15-His protein
RRDASGDLLNTEAHSAPAQRWSMQVPAEVNAEAGDAAVLPCTFTHPHRHYDGPLTAIWRSGEPYAGPQVFRCTAAPGSELCQTALSLHGRFRLLGNPRRNDLSLRVERLALADSGRYFCRVEFTGDAHDRYESRHGVRLRVTAAAPRIVNISVLPGPAHAFRALCTAEGEPPPALAWSGPAPGNSSAALQGQGHGYQVTAELPALTRDGRYTCTAANSLGRAEASVYLFRFHGAPGTSTGGGSGGGSHHHHHHHHHH

SEQ ID NO: 81 - protein, 15 aa, Artificial Sequence
  21F6C6-hH2L4V LCDR1
RASQSVDYEGDSYMN

SEQ ID NO: 82 - protein, 111 aa, Artificial Sequence
  21F6C6-hH2L4V Light Chain Variable Region
DIQMTQSPSSLSASVGDRVTITCRASQSVDYEGDSYMNWYQQKPGKAPKLLIYAASNLQSGVPSRFSGSGSGTDFTLTISSLQPEDFATYYCQQSNEAPLTFGQGTKLEIK